European Patent Application EP 4 282 950 A1, published November 29, 2023. Title: ENTEROCOCCUS FAECIUM, DRUG FOR PREVENTING OR TREATING TUMOR, AND APPLICATION. Applicant: MOON (GUANGZHOU) BIOTECH CO., LTD. The sequence listing filed with the application follows.

SEQUENCE LISTING (1 sequence)

SEQ ID NO: 1 - DNA, 1424 bp, Artificial Sequence
tgcaagtcgtacgcttctttttccaccggagcttgctccaccggaaaaagaggagtggcgaacgggtgagtaacacgtgggtaacctgcccatcagaaggggataacacttggaaacaggtgctaataccgtataacaatcgaaaccgcatggttttgatttgaaaggcgctttcgggtgtcgctgatggatggacccgcggtgcattagctagttggtgaggtaacggctcaccaaggccacgatgcatagccgacctgagagggtgatcggccacattgggactgagacacggcccaaactcctacgggaggcagcagtagggaatcttcggcaatggacgaaagtctgaccgagcaacgccgcgtgagtgaagaaggttttcggatcgtaaaactctgttgttagagaagaacaaggatgagagtaactgttcatcccttgacggtatctaaccagaaagccacggctaactacgtgccagcagccgcggtaatacgtaggtggcaagcgttgtccggatttattgggcgtaaagcgagcgcaggcggtttcttaagtctgatgtgaaagcccccggctcaaccggggagggtcattggaaactgggagacttgagtgcagaagaggagagtggaattccatgtgtagcggtgaaatgcgtagatatatggaggaacaccagtggcgaaggcggctctctggtctgtaactgacgctgaggctcgaaagcgtggggagcaaacaggattagataccctggtagtccacgccgtaaacgatgagtgctaagtgttggagggtttccgcccttcagtgctgcagctaacgcattaagcactccgcctggggagtacgaccgcaaggttgaaactcaaaggaattgacgggggcccgcacaagcggtggagcatgtggtttaattcgaagcaacgcgaagaaccttaccaggtcttgacatcctttgaccactctagagatagagcttccccttcgggggcaaagtgacaggtggtgcatggttgtcgtcagctcgtgtcgtgagatgttgggttaagtcccgcaacgagcgcaacccttattgttagttgccatcattcagttgggcactctagcaagactgccggtgacaaaccggaggaaggtggggatgacgtcaaatcatcatgccccttatgacctgggctacacacgtgctacaatgggaagtacaacgagttgcgaagtcgcgaggctaagctaatctcttaaagcttctctcagttcggattgcaggctgcaactcgcctgcatgaagccggaatcgctagtaatcgcggatcagcacgccgcggtgaatacgttcccgggccttgtacacaccgcccgtcacaccacgagagtttgtaacacccgaagtcggtgaggtaacctttttggagcca